European Patent Specification EP 3 575 322 B1, published November 27, 2024. Title: ANTI-PD-1 MONOCLONAL ANTIBODY, AND PREPARATION METHOD THEREFOR AND APPLICATION THEREFOR. Applicant: SUNSHINE GUOJIAN PHARMACEUTICAL (SHANGHAI) CO., LTD. The sequence listing filed with the application follows.

SEQUENCE LISTING (40 sequences)

SEQ ID NO: 1 - protein, 5 aa, Artificial
  A sequence of CDRH1
SYDMS

SEQ ID NO: 2 - protein, 17 aa, Artificial
  A sequence of CDRH2
TISGGGRYTYYPDTVKG

SEQ ID NO: 3 - protein, 8 aa, Artificial
  A sequence of CDRH3
PYGGYFDV

SEQ ID NO: 4 - protein, 11 aa, Artificial
  A sequence of CDRL1
RASQSISNFLH

SEQ ID NO: 5 - protein, 7 aa, Artificial
  A sequence of CDRL2
YASQSIS

SEQ ID NO: 6 - protein, 9 aa, Artificial
  A sequence of CDRL3
QQSNSWPHT

SEQ ID NO: 7 - protein, 117 aa, Artificial
  Heavy chain variable region amino acid sequence of mAb1-25-Humanized
EVKLVESGGGLVQPGGSLRLSCAASGFAFSSYDMSWVRQAPGKRLEWVATISGGGRYTYYPDTVKGRFTISRDNAKNSHYLQMNSLRAEDTAVYFCASPYGGYFDVWGQGTLVTVSS

SEQ ID NO: 8 - protein, 444 aa, Artificial
  Heavy chain full length amino acid sequence of mAb1-25-Humanized
EVKLVESGGGLVQPGGSLRLSCAASGFAFSSYDMSWVRQAPGKRLEWVATISGGGRYTYYPDTVKGRFTISRDNAKNSHYLQMNSLRAEDTAVYFCASPYGGYFDVWGQGTLVTVSSASTKGPSVFPLAPCSRSTSESTAALGCLVKDYFPEPVTVSWNSGALTSGVHTFPAVLQSSGLYSLSSVVTVPSSSLGTKTYTCNVDHKPSNTKVDKRVESKYGPPCPPCPAPEFLGGPSVFLFPPKPKDTLMISRTPEVTCVVVDVSQEDPEVQFNWYVDGVEVHNAKTKPREEQFNSTYRVVSVLTVLHQDWLNGKEYKCKVSNKGLPSSIEKTISKAKGQPREPQVYTLPPSQEEMTKNQVSLTCLVKGFYPSDIAVEWESNGQPENNYKTTPPVLDSDGSFFLYSRLTVDKSRWQEGNVFSCSVMHEALHNHYTQKSLSLSLGK

SEQ ID NO: 9 - protein, 107 aa, Artificial
  Light chain variable region amino acid sequence of mAb1-25-Humanized
EIVLTQSPATLSLSPGERATLSCRASQSISNFLHWYQQKPGQAPRLLIKYASQSISGIPARFSGSGSGTDFTLTISSLEPEDFAVYFCQQSNSWPHTFGQGTKVEIK

SEQ ID NO: 10 - protein, 214 aa, Artificial
  Light chain full length amino acid sequence of mAb1-25-Humanized
EIVLTQSPATLSLSPGERATLSCRASQSISNFLHWYQQKPGQAPRLLIKYASQSISGIPARFSGSGSGTDFTLTISSLEPEDFAVYFCQQSNSWPHTFGQGTKVEIKRTVAAPSVFIFPPSDEQLKSGTASVVCLLNNFYPREAKVQWKVDNALQSGNSQESVTEQDSKDSTYSLSSTLTLSKADYEKHKVYACEVTHQGLSSPVTKSFNRGEC

SEQ ID NO: 11 - DNA, 1332 bp, Artificial
  Heavy chain nucleotide sequence of mAb1-25-Humanized
gaagtcaaactcgtggagtccggcggaggcctcgttcaaccaggtggatctcttcgtttgtcctgcgcagcatcaggattcgctttctccagctacgacatgagctgggtccgacaggctcctggaaagaggctggaatgggttgctactatcagcggcggtggtagatatacttattaccccgataccgtaaaggggaggttcaccattagtcgcgataacgccaaaaattcacactacctgcagatgaactctctgcgggccgaggacaccgccgtgtacttttgtgccagtccctatggcgggtattttgacgtgtggggccaggggacactggtgactgtgagttctgcaagtaccaagggacctagtgttttccctcttgcaccttgctccaggtcaacatcagagtccacagctgctcttggatgtctcgttaaggactacttcccagagccagttaccgtatcctggaactccggagctttgacaagcggcgttcatacattcccagctgtgttgcagagttctgggttgtacagtttgagctcagtggtgaccgtgccttcatcttctttgggcactaagacctacacctgcaacgtggatcacaagccaagcaacaccaaggtggataagagggtggagtccaagtacggcccaccatgtcctccatgtccagcccctgaatttttgggcgggccttctgtctttctgtttcctcctaaacctaaagataccctgatgatcagccgcacacccgaagtcacttgtgtggtcgtggatgtgtctcaggaagatcccgaagtgcagtttaactggtatgtcgatggcgtggaagtgcataatgccaaaactaagccccgcgaagaacagttcaacagcacttatcgggtcgtgtctgtgctcacagtcctccatcaggattggctgaatgggaaagaatataagtgcaaggtgagcaataagggcctccccagcagcatcgagaagactattagcaaagccaaagggcagccacgggaaccccaggtgtacactctgcccccctctcaggaggagatgactaaaaatcaggtctctctgacttgtctggtgaaagggttttatcccagcgacattgccgtggagtgggagtctaatggccagcccgagaataattataagacaactccccccgtcctggactctgacggcagctttttcctgtattctcggctgacagtggacaaaagtcgctggcaggagggcaatgtctttagttgcagtgtcatgcatgaggccctgcacaatcactatacacagaaaagcctgtctctgagtctgggcaaa

SEQ ID NO: 12 - DNA, 642 bp, Artificial
  Light chain nucleotide sequence of mAb1-25-Humanized
gagatcgtccttacccaatcaccagcaaccttgtcactgtcaccaggtgaaagagcaaccctcagttgtagggctagtcagagtatctccaacttcctgcactggtaccagcagaagcctggacaggcccctcggttgctcattaagtacgcctctcaatctatcagcggaatccccgctcgcttttctggctctggctccgggactgatttcactctgacaatttccagcctggaacccgaggactttgccgtttatttttgccagcagagcaatagctggccccatacattcgggcagggcacaaaagtggagataaaacgcactgtggctgcccccagtgttttcatatttccccccagtgatgagcaactgaagtccggcacagcctctgttgtatgtctgctgaataatttttatccacgggaggccaaggtgcagtggaaggtggacaatgccctgcagtctgggaactctcaagagagtgtgacagagcaggacagtaaagacagcacctatagcctcagcagcaccctgaccctgtctaaagccgactatgaaaaacacaaagtgtatgcctgcgaagtgacccatcaggggctcagctctcccgttaccaagagctttaaccgaggcgaatgt

SEQ ID NO: 13 - protein, 5 aa, Artificial
  Another sequence of CDRH1
SYDMS

SEQ ID NO: 14 - protein, 17 aa, Artificial
  Another sequence of CDRH2
TISGGGRYTYYPDSVKG

SEQ ID NO: 15 - protein, 9 aa, Artificial
  Another sequence of CDRH3
RYDVDWFAY

SEQ ID NO: 16 - protein, 11 aa, Artificial
  Another sequence of CDRL1
RASQSISNNLH

SEQ ID NO: 17 - protein, 7 aa, Artificial
  Another sequence of CDRL2
YASQSIS

SEQ ID NO: 18 - protein, 9 aa, Artificial
  Another sequence of CDRL3
QQSNSWPLT

SEQ ID NO: 19 - protein, 118 aa, Artificial
  Heavy chain variable region amino acid sequence of mAb1-15-humanized
EVQLVESGGGLVQPGGSLRLSCAASGFTFSSYDMSWVRQAPGKRLEWVATISGGGRYTYYPDSVKGRFTISRDNAKNSLYLQMNSLRAEDTAVYYCANRYDVDWFAYWGQGTLVTVSS

SEQ ID NO: 20 - protein, 445 aa, Artificial
  Heavy chain full length amino acid sequence of mAb1-15-humanized
EVQLVESGGGLVQPGGSLRLSCAASGFTFSSYDMSWVRQAPGKRLEWVATISGGGRYTYYPDSVKGRFTISRDNAKNSLYLQMNSLRAEDTAVYYCANRYDVDWFAYWGQGTLVTVSSASTKGPSVFPLAPCSRSTSESTAALGCLVKDYFPEPVTVSWNSGALTSGVHTFPAVLQSSGLYSLSSVVTVPSSSLGTKTYTCNVDHKPSNTKVDKRVESKYGPPCPPCPAPEFLGGPSVFLFPPKPKDTLMISRTPEVTCVVVDVSQEDPEVQFNWYVDGVEVHNAKTKPREEQFNSTYRVVSVLTVLHQDWLNGKEYKCKVSNKGLPSSIEKTISKAKGQPREPQVYTLPPSQEEMTKNQVSLTCLVKGFYPSDIAVEWESNGQPENNYKTTPPVLDSDGSFFLYSRLTVDKSRWQEGNVFSCSVMHEALHNHYTQKSLSLSLGK

SEQ ID NO: 21 - protein, 107 aa, Artificial
  Light chain variable region amino acid sequence of mAb1-15-humanized
EIVLTQSPATLSLSPGERATLSCRASQSISNNLHWYQQKPGQAPRLLIKYASQSISGIPARFSGSGSGTDFTLTISSLEPEDFAVYFCQQSNSWPLTFGQGTKVEIK

SEQ ID NO: 22 - protein, 214 aa, Artificial
  Light chain full length amino acid sequence of mAb1-15-humanized
EIVLTQSPATLSLSPGERATLSCRASQSISNNLHWYQQKPGQAPRLLIKYASQSISGIPARFSGSGSGTDFTLTISSLEPEDFAVYFCQQSNSWPLTFGQGTKVEIKRTVAAPSVFIFPPSDEQLKSGTASVVCLLNNFYPREAKVQWKVDNALQSGNSQESVTEQDSKDSTYSLSSTLTLSKADYEKHKVYACEVTHQGLSSPVTKSFNRGEC

SEQ ID NO: 23 - DNA, 354 bp, Artificial
  Heavy chain variable region nucleotide sequence of mAb1-15
gaagtgaacctggtggagtctgggggaggcttagtgaagcctggagggtccctgaaactctcctgtgcagcctctggattcactttcagtagctatgacatgtcttgggttcgccagactccggagaagaggctggagtgggtcgcaaccattagtggtggtggtcgttacacctattatccagacagtgtgaaggggcgattcaccatctccagagacaatgccaagaacaacctgtacctgcaaatgagcagtctgaggtctgaggacacggccttgtattactgtgcaaataggtacgacgtggactggtttgcttactggggccaagggactctggtcactgtctctgca

SEQ ID NO: 24 - protein, 118 aa, Artificial
  Heavy chain variable region amino acid sequence of mAb1-15
EVNLVESGGGLVKPGGSLKLSCAASGFTFSSYDMSWVRQTPEKRLEWVATISGGGRYTYYPDSVKGRFTISRDNAKNNLYLQMSSLRSEDTALYYCANRYDVDWFAYWGQGTLVTVSA

SEQ ID NO: 25 - DNA, 321 bp, Artificial
  Light chain variable region nucleotide sequence of mAb1-15
gatattgtgctaactcagtctccagccaccctgtctgtgactccaggagatagcgtcagtctttcctgcagggccagccaaagtattagcaacaacctacactggtatcaacaaaaatcacatgagtctccaaggcttctcatcaagtatgcttcccagtccatctctgggatcccctccaggttcagtggtagtggatcagggacagatttcactctcagtatcaacagtgtggagactgaagattttggaatgtatttctgtcaacagagtaacagctggccgctcacgttcggtgctgggaccaagctggagctgaat

SEQ ID NO: 26 - protein, 107 aa, Artificial
  Light chain variable region amino acid sequence of mAb1-15
DIVLTQSPATLSVTPGDSVSLSCRASQSISNNLHWYQQKSHESPRLLIKYASQSISGIPSRFSGSGSGTDFTLSINSVETEDFGMYFCQQSNSWPLTFGAGTKLELN

SEQ ID NO: 27 - DNA, 351 bp, Artificial
  Heavy chain variable region nucleotide sequence of mAb1-25
gaagtgaagctggtggagtctgggggagacttagtgaagcctggagggtccctgaaactctcctgtgtagcctctggattcgctttcagtagctatgacatgtcttgggttcgccaaactccggagaagcggctggagtgggtcgctaccattagtggtggtggtcgttacacctactatccagacactgtgaagggccgattcaccatctccagagacaatgccaggaacacccactacctgcaaatgagcagtctgaggtctgaggacacggccctctatttttgtgcaagtccttacggcggttacttcgatgtctggggcgcagggaccacggtcaccgtctcctca

SEQ ID NO: 28 - protein, 117 aa, Artificial
  Heavy chain variable region amino acid sequence of mAb1-25
EVKLVESGGDLVKPGGSLKLSCVASGFAFSSYDMSWVRQTPEKRLEWVATISGGGRYTYYPDTVKGRFTISRDNARNTHYLQMSSLRSEDTALYFCASPYGGYFDVWGAGTTVTVSS

SEQ ID NO: 29 - DNA, 321 bp, Artificial
  Light chain variable region nucleotide sequence of mAb1-25
gatattgtgctaactcagtctccagccaccctgtctgtgactccgggagctagagtcagtctttcctgcagggccagtcaaagtattagcaacttcctacactggtatcaacaaaaatcacatgagtctccaaggcttctcatcaaatatgcttctcagtccatttctgggatcccctccaggttcagtggcagtggatcagggacagatttcactctcagtatcagcagtgtggagactgaagattttggaatgtatttctgtcaacagagtaacagctggcctcatacgttcggtgctgggaccaagctggagctgaaa

SEQ ID NO: 30 - protein, 107 aa, Artificial
  Light chain variable region amino acid sequence of mAb1-25
DIVLTQSPATLSVTPGARVSLSCRASQSISNFLHWYQQKSHESPRLLIKYASQSISGIPSRFSGSGSGTDFTLSISSVETEDFGMYFCQQSNSWPHTFGAGTKLELK

SEQ ID NO: 31 - DNA, 354 bp, Artificial
  Heavy chain variable region nucleotide sequence of mAb1-15-humanized
gaggtgcagctggtggagagcggcggcggcctggtgcagcccggcggcagcctgaggctgagctgcgccgccagcggcttcaccttcagcagctacgacatgagctgggtgaggcaggcccccggcaagaggctggagtgggtggccaccatcagcggcggcggcaggtacacctactaccccgacagcgtgaagggcaggttcaccatcagcagggacaacgccaagaacagcctgtacctgcagatgaacagcctgagggccgaggacaccgccgtgtactactgcgccaacaggtacgacgtggactggttcgcctactggggccagggcaccctggtgaccgtgagcagc

SEQ ID NO: 32 - DNA, 321 bp, Artificial
  Light chain variable region nucleotide sequence of mAb1-15-humanized
gagatcgtgctgacccagagccccgccaccctgagcctgagccccggcgagagggccaccctgagctgcagggccagccagagcatcagcaacaacctgcactggtaccagcagaagcccggccaggcccccaggctgctgatcaagtacgccagccagagcatcagcggcatccccgccaggttcagcggcagcggcagcggcaccgacttcaccctgaccatcagcagcctggagcccgaggacttcgccgtgtacttctgccagcagagcaacagctggcccctgaccttcggccagggcaccaaggtggagatcaag

SEQ ID NO: 33 - DNA, 351 bp, Artificial
  Heavy chain variable region nucleotide sequence of mAb1-25-Humanized
gaagtcaaactcgtggagtccggcggaggcctcgttcaaccaggtggatctcttcgtttgtcctgcgcagcatcaggattcgctttctccagctacgacatgagctgggtccgacaggctcctggaaagaggctggaatgggttgctactatcagcggcggtggtagatatacttattaccccgataccgtaaaggggaggttcaccattagtcgcgataacgccaaaaattcacactacctgcagatgaactctctgcgggccgaggacaccgccgtgtacttttgtgccagtccctatggcgggtattttgacgtgtggggccaggggacactggtgactgtgagttct

SEQ ID NO: 34 - DNA, 321 bp, Artificial
  Light chain variable region nucleotide sequence of mAb1-25-Humanized
gagatcgtccttacccaatcaccagcaaccttgtcactgtcaccaggtgaaagagcaaccctcagttgtagggctagtcagagtatctccaacttcctgcactggtaccagcagaagcctggacaggcccctcggttgctcattaagtacgcctctcaatctatcagcggaatccccgctcgcttttctggctctggctccgggactgatttcactctgacaatttccagcctggaacccgaggactttgccgtttatttttgccagcagagcaatagctggccccatacattcgggcagggcacaaaagtggagataaaa

SEQ ID NO: 35 - DNA, 981 bp, Artificial
  Nucleotide sequence of human immunoglobulin IgG4 constant region
gcaagtaccaagggacctagtgttttccctcttgcaccttgctccaggtcaacatcagagtccacagctgctcttggatgtctcgttaaggactacttcccagagccagttaccgtatcctggaactccggagctttgacaagcggcgttcatacattcccagctgtgttgcagagttctgggttgtacagtttgagctcagtggtgaccgtgccttcatcttctttgggcactaagacctacacctgcaacgtggatcacaagccaagcaacaccaaggtggataagagggtggagtccaagtacggcccaccatgtcctccatgtccagcccctgaatttttgggcgggccttctgtctttctgtttcctcctaaacctaaagataccctgatgatcagccgcacacccgaagtcacttgtgtggtcgtggatgtgtctcaggaagatcccgaagtgcagtttaactggtatgtcgatggcgtggaagtgcataatgccaaaactaagccccgcgaagaacagttcaacagcacttatcgggtcgtgtctgtgctcacagtcctccatcaggattggctgaatgggaaagaatataagtgcaaggtgagcaataagggcctccccagcagcatcgagaagactattagcaaagccaaagggcagccacgggaaccccaggtgtacactctgcccccctctcaggaggagatgactaaaaatcaggtctctctgacttgtctggtgaaagggttttatcccagcgacattgccgtggagtgggagtctaatggccagcccgagaataattataagacaactccccccgtcctggactctgacggcagctttttcctgtattctcggctgacagtggacaaaagtcgctggcaggagggcaatgtctttagttgcagtgtcatgcatgaggccctgcacaatcactatacacagaaaagcctgtctctgagtctgggcaaa

SEQ ID NO: 36 - protein, 327 aa, Artificial
  Amino acid sequence of human immunoglobulin IgG4 constant region
ASTKGPSVFPLAPCSRSTSESTAALGCLVKDYFPEPVTVSWNSGALTSGVHTFPAVLQSSGLYSLSSVVTVPSSSLGTKTYTCNVDHKPSNTKVDKRVESKYGPPCPPCPAPEFLGGPSVFLFPPKPKDTLMISRTPEVTCVVVDVSQEDPEVQFNWYVDGVEVHNAKTKPREEQFNSTYRVVSVLTVLHQDWLNGKEYKCKVSNKGLPSSIEKTISKAKGQPREPQVYTLPPSQEEMTKNQVSLTCLVKGFYPSDIAVEWESNGQPENNYKTTPPVLDSDGSFFLYSRLTVDKSRWQEGNVFSCSVMHEALHNHYTQKSLSLSLGK

SEQ ID NO: 37 - DNA, 1335 bp, Artificial
  Heavy chain full length nucleotide sequence of mAb1-15-Humanized
gaggtgcagctggtggagagcggcggcggcctggtgcagcccggcggcagcctgaggctgagctgcgccgccagcggcttcaccttcagcagctacgacatgagctgggtgaggcaggcccccggcaagaggctggagtgggtggccaccatcagcggcggcggcaggtacacctactaccccgacagcgtgaagggcaggttcaccatcagcagggacaacgccaagaacagcctgtacctgcagatgaacagcctgagggccgaggacaccgccgtgtactactgcgccaacaggtacgacgtggactggttcgcctactggggccagggcaccctggtgaccgtgagcagcgcaagtaccaagggacctagtgttttccctcttgcaccttgctccaggtcaacatcagagtccacagctgctcttggatgtctcgttaaggactacttcccagagccagttaccgtatcctggaactccggagctttgacaagcggcgttcatacattcccagctgtgttgcagagttctgggttgtacagtttgagctcagtggtgaccgtgccttcatcttctttgggcactaagacctacacctgcaacgtggatcacaagccaagcaacaccaaggtggataagagggtggagtccaagtacggcccaccatgtcctccatgtccagcccctgaatttttgggcgggccttctgtctttctgtttcctcctaaacctaaagataccctgatgatcagccgcacacccgaagtcacttgtgtggtcgtggatgtgtctcaggaagatcccgaagtgcagtttaactggtatgtcgatggcgtggaagtgcataatgccaaaactaagccccgcgaagaacagttcaacagcacttatcgggtcgtgtctgtgctcacagtcctccatcaggattggctgaatgggaaagaatataagtgcaaggtgagcaataagggcctccccagcagcatcgagaagactattagcaaagccaaagggcagccacgggaaccccaggtgtacactctgcccccctctcaggaggagatgactaaaaatcaggtctctctgacttgtctggtgaaagggttttatcccagcgacattgccgtggagtgggagtctaatggccagcccgagaataattataagacaactccccccgtcctggactctgacggcagctttttcctgtattctcggctgacagtggacaaaagtcgctggcaggagggcaatgtctttagttgcagtgtcatgcatgaggccctgcacaatcactatacacagaaaagcctgtctctgagtctgggcaaa

SEQ ID NO: 38 - DNA, 321 bp, Artificial
  Nucleotide sequence of human immunoglobulin Kappa chain constant region
cgcactgtggctgcccccagtgttttcatatttccccccagtgatgagcaactgaagtccggcacagcctctgttgtatgtctgctgaataatttttatccacgggaggccaaggtgcagtggaaggtggacaatgccctgcagtctgggaactctcaagagagtgtgacagagcaggacagtaaagacagcacctatagcctcagcagcaccctgaccctgtctaaagccgactatgaaaaacacaaagtgtatgcctgcgaagtgacccatcaggggctcagctctcccgttaccaagagctttaaccgaggcgaatgt

SEQ ID NO: 39 - protein, 107 aa, Artificial [sequence omitted]

SEQ ID NO: 40 - DNA, 642 bp, Artificial
  Light chain full length nucleotide sequence of mAb1-15-Humanized
gagatcgtgctgacccagagccccgccaccctgagcctgagccccggcgagagggccaccctgagctgcagggccagccagagcatcagcaacaacctgcactggtaccagcagaagcccggccaggcccccaggctgctgatcaagtacgccagccagagcatcagcggcatccccgccaggttcagcggcagcggcagcggcaccgacttcaccctgaccatcagcagcctggagcccgaggacttcgccgtgtacttctgccagcagagcaacagctggcccctgaccttcggccagggcaccaaggtggagatcaagcgcactgtggctgcccccagtgttttcatatttccccccagtgatgagcaactgaagtccggcacagcctctgttgtatgtctgctgaataatttttatccacgggaggccaaggtgcagtggaaggtggacaatgccctgcagtctgggaactctcaagagagtgtgacagagcaggacagtaaagacagcacctatagcctcagcagcaccctgaccctgtctaaagccgactatgaaaaacacaaagtgtatgcctgcgaagtgacccatcaggggctcagctctcccgttaccaagagctttaaccgaggcgaatgt